European Patent Application EP 4 527 857 A1, published March 26, 2025. Title: BIFUNCTIONAL PROTEIN, AND PREPARATION THEREOF AND USE THEREOF. Applicant: Suzhou Transcenta therapeutics Co.,Ltd. Application WO. The sequence listing filed with the application follows.

SEQUENCE LISTING (122 sequences)

SEQ ID NO: 1 - protein, 5 aa, synthetic construct
  REGION 1..5: note = Synthetic
DYYMN

SEQ ID NO: 2 - protein, 17 aa, synthetic construct
  REGION 1..17: note = Synthetic
DINPNNGGTSYNHKFKG

SEQ ID NO: 3 - protein, 8 aa, synthetic construct
  REGION 1..8: note = Synthetic
WGDGPFAY

SEQ ID NO: 4 - protein, 11 aa, synthetic construct
  REGION 1..11: note = Synthetic
KASQNVGAAVA

SEQ ID NO: 5 - protein, 7 aa, synthetic construct
  REGION 1..7: note = Synthetic
SASNRYT

SEQ ID NO: 6 - protein, 8 aa, synthetic construct
  REGION 1..8: note = Synthetic
QQYSNYPT

SEQ ID NO: 7 - protein, 11 aa, synthetic construct
  REGION 1..11: note = Synthetic
KASQNVGAIVA

SEQ ID NO: 8 - protein, 11 aa, synthetic construct
  REGION 1..11: note = Synthetic
KASQNVPAAVA

SEQ ID NO: 9 - protein, 11 aa, synthetic construct
  REGION 1..11: note = Synthetic
KASQNVKGAVA

SEQ ID NO: 10 - protein, 7 aa, synthetic construct
  REGION 1..7: note = Synthetic
SNSHRYT

SEQ ID NO: 11 - protein, 7 aa, synthetic construct
  REGION 1..7: note = Synthetic
SRSVRYT

SEQ ID NO: 12 - protein, 7 aa, synthetic construct
  REGION 1..7: note = Synthetic
SVSDRYT

SEQ ID NO: 13 - protein, 17 aa, synthetic construct
  REGION 1..17: note = Synthetic
DINPNNADTMYNHKFKG

SEQ ID NO: 14 - protein, 17 aa, synthetic construct
  REGION 1..17: note = Synthetic
DINPNNAQTQYNHKFKG

SEQ ID NO: 15 - protein, 17 aa, synthetic construct
  REGION 1..17: note = Synthetic
DINPNNAETLYNHKFKG

SEQ ID NO: 16 - protein, 17 aa, synthetic construct
  REGION 1..17: note = Synthetic
DINPNNGLTSYNHKFKG

SEQ ID NO: 17 - protein, 17 aa, synthetic construct
  REGION 1..17: note = Synthetic
DINPNNAQTVYNHKFKG

SEQ ID NO: 18 - protein, 17 aa, synthetic construct
  REGION 1..17: note = Synthetic
DINPNNAGTSYNHKFKG

SEQ ID NO: 19 - protein, 17 aa, synthetic construct
  REGION 1..17: note = Synthetic
  REGION 7..8: note = misc_feature - Xaa can be any naturally occurring amino acid
  SITE 10: note = misc_feature - Xaa can be any naturally occurring amino acid
DINPNNXXTXYNHKFKG

SEQ ID NO: 20 - protein, 11 aa, synthetic construct
  REGION 1..11: note = Synthetic
  REGION 7..9: note = misc_feature - Xaa can be any naturally occurring amino acid
KASQNVXXXVA

SEQ ID NO: 21 - protein, 7 aa, synthetic construct
  REGION 1..7: note = Synthetic
  SITE 2: note = misc_feature - Xaa can be any naturally occurring amino acid
  SITE 4: note = misc_feature - Xaa can be any naturally occurring amino acid
SXSXRYT

SEQ ID NO: 22 - protein, 30 aa, synthetic construct
  REGION 1..30: note = Synthetic
QVQLVQSGAEVKKPGASVKVSCKASGYTFT

SEQ ID NO: 23 - protein, 14 aa, synthetic construct
  REGION 1..14: note = Synthetic
WVRQAPGQGLEWMG

SEQ ID NO: 24 - protein, 32 aa, synthetic construct
  REGION 1..32: note = Synthetic
RVTMTRDTSISTAYMELSRLRSDDTAVYYCAR

SEQ ID NO: 25 - protein, 11 aa, synthetic construct
  REGION 1..11: note = Synthetic
WGQGTLVTVSS

SEQ ID NO: 26 - protein, 23 aa, synthetic construct
  REGION 1..23: note = Synthetic
DIQMTQSPSSLSASVGDRVTITC

SEQ ID NO: 27 - protein, 15 aa, synthetic construct
  REGION 1..15: note = Synthetic
WYQQKPGKAPKLLIY

SEQ ID NO: 28 - protein, 32 aa, synthetic construct
  REGION 1..32: note = Synthetic
GVPSRFSGSGSGTDFTFTISSLQPEDIATYYC

SEQ ID NO: 29 - protein, 10 aa, synthetic construct
  REGION 1..10: note = Synthetic
FGQGTKLEIK

SEQ ID NO: 30 - protein, 30 aa, synthetic construct
  REGION 1..30: note = Synthetic
QVQLVQSGAEVKKPGASVKVSCKASGYVFT

SEQ ID NO: 31 - protein, 14 aa, synthetic construct
  REGION 1..14: note = Synthetic
WVRQAPGQSLEWMG

SEQ ID NO: 32 - protein, 32 aa, synthetic construct
  REGION 1..32: note = Synthetic
RVTVTVDTSISTAYMELSRLRSDDTAVYYCAR

SEQ ID NO: 33 - protein, 32 aa, synthetic construct
  REGION 1..32: note = Synthetic
RVTVTVDTSISTAYMELSRLRSDDTAVYYCVK

SEQ ID NO: 34 - protein, 32 aa, synthetic construct
  REGION 1..32: note = Synthetic
RVTVTVDKSISTAYMELSRLRSDDTAVYYCAR

SEQ ID NO: 35 - protein, 32 aa, synthetic construct
  REGION 1..32: note = Synthetic
RVTVTVDKSISTAYMELSRLRSDDTAVYYCVK

SEQ ID NO: 36 - protein, 15 aa, synthetic construct
  REGION 1..15: note = Synthetic
WYQQKPGKSPKLLIY

SEQ ID NO: 37 - protein, 32 aa, synthetic construct
  REGION 1..32: note = Synthetic
GVPSRFSGSGSGTDFTLTISSLQPEDIATYYC

SEQ ID NO: 38 - protein, 32 aa, synthetic construct
  REGION 1..32: note = Synthetic
GVPDRFSGSGSGTDFTLTISSLQPEDIATYYC

SEQ ID NO: 39 - protein, 32 aa, synthetic construct; identical to SEQ ID NO: 37
  REGION 1..32: note = Synthetic

SEQ ID NO: 40 - protein, 30 aa, synthetic construct
  REGION 1..30: note = Synthetic
  SITE 28: note = misc_feature - Xaa can be any naturally occurring amino acid
QVQLVQSGAEVKKPGASVKVSCKASGYXFT

SEQ ID NO: 41 - protein, 14 aa, synthetic construct
  REGION 1..14: note = Synthetic
  SITE 9: note = misc_feature - Xaa can be any naturally occurring amino acid
WVRQAPGQXLEWMG

SEQ ID NO: 42 - protein, 32 aa, synthetic construct
  REGION 1..32: note = Synthetic
  SITE 4: note = misc_feature - Xaa can be any naturally occurring amino acid
  SITE 8: note = misc_feature - Xaa can be any naturally occurring amino acid
  REGION 31..32: note = misc_feature - Xaa can be any naturally occurring amino acid
RVTXTVDXSISTAYMELSRLRSDDTAVYYCXX

SEQ ID NO: 43 - protein, 15 aa, synthetic construct
  REGION 1..15: note = Synthetic
  SITE 9: note = misc_feature - Xaa can be any naturally occurring amino acid
WYQQKPGKXPKLLIY

SEQ ID NO: 44 - protein, 32 aa, synthetic construct
  REGION 1..32: note = Synthetic
  SITE 4: note = misc_feature - Xaa can be any naturally occurring amino acid
  SITE 17: note = misc_feature - Xaa can be any naturally occurring amino acid
GVPXRFSGSGSGTDFTXTISSLQPEDIATYYC

SEQ ID NO: 45 - protein, 32 aa, synthetic construct; identical to SEQ ID NO: 38
  REGION 1..32: note = Synthetic

SEQ ID NO: 46 - protein, 117 aa, synthetic construct
  REGION 1..117: note = Synthetic
EVQLQQSGPELVKPGASVKISCKASGYVFTDYYMNWVKQSHGKSLEWIGDINPNNGGTSYNHKFKGKATVTVDKSSRTAYMELLSLTSEDSAVYYCVKWGDGPFAYWGQGTLVTVSA

SEQ ID NO: 47 - protein, 106 aa, synthetic construct
  REGION 1..106: note = Synthetic
DIVMTQSQKFMSTSVGDRVSITCKASQNVGAAVAWYQQKPGQSPKLLIYSASNRYTGVPDRFTGSGSGTDFTLTISNMQSEDLADYFCQQYSNYPTFGSGTKLGIK

SEQ ID NO: 48 - protein, 98 aa, Homo sapiens
QVQLVQSGAEVKKPGASVKVSCKASGYTFTGYYMHWVRQAPGQGLEWMGWINPNSGGTNYAQKFQGRVTMTRDTSISTAYMELSRLRSDDTAVYYCAR

SEQ ID NO: 49 - protein, 117 aa, synthetic construct
  REGION 1..117: note = Synthetic
QVQLVQSGAEVKKPGASVKVSCKASGYTFTDYYMNWVRQAPGQGLEWMGDINPNNGGTSYNHKFKGRVTVTVDTSISTAYMELSRLRSDDTAVYYCARWGDGPFAYWGQGTLVTVSS

SEQ ID NO: 50 - protein, 117 aa, synthetic construct
  REGION 1..117: note = Synthetic
QVQLVQSGAEVKKPGASVKVSCKASGYTFTDYYMNWVRQAPGQGLEWMGDINPNNGGTSYNHKFKGRVTVTVDTSISTAYMELSRLRSDDTAVYYCVKWGDGPFAYWGQGTLVTVSS

SEQ ID NO: 51 - protein, 117 aa, synthetic construct
  REGION 1..117: note = Synthetic
QVQLVQSGAEVKKPGASVKVSCKASGYVFTDYYMNWVRQAPGQGLEWMGDINPNNGGTSYNHKFKGRVTVTVDKSISTAYMELSRLRSDDTAVYYCARWGDGPFAYWGQGTLVTVSS

SEQ ID NO: 52 - protein, 117 aa, synthetic construct
  REGION 1..117: note = Synthetic
QVQLVQSGAEVKKPGASVKVSCKASGYVFTDYYMNWVRQAPGQSLEWMGDINPNNGGTSYNHKFKGRVTVTVDKSISTAYMELSRLRSDDTAVYYCVKWGDGPFAYWGQGTLVTVSS

SEQ ID NO: 53 - protein, 95 aa, synthetic construct
  REGION 1..95: note = Synthetic
DIQMTQSPSSLSASVGDRVTITCQASQDISNYLNWYQQKPGKAPKLLIYDASNLETGVPSRFSGSGSGTDFTFTISSLQPEDIATYYCQQYDNLP

SEQ ID NO: 54 - protein, 106 aa, synthetic construct
  REGION 1..106: note = Synthetic
DIQMTQSPSSLSASVGDRVTITCKASQNVGAAVAWYQQKPGKAPKLLIYSASNRYTGVPSRFSGSGSGTDFTLTISSLQPEDIATYYCQQYSNYPTFGQGTKLEIK

SEQ ID NO: 55 - protein, 106 aa, synthetic construct
  REGION 1..106: note = Synthetic
DIQMTQSPSSLSASVGDRVTITCKASQNVGAAVAWYQQKPGKSPKLLIYSASNRYTGVPDRFSGSGSGTDFTLTISSLQPEDIATYYCQQYSNYPTFGQGTKLEIK

SEQ ID NO: 56 - protein, 117 aa, synthetic construct
  REGION 1..117: note = Synthetic
QVQLVQSGAEVKKPGASVKVSCKASGYVFTDYYMNWVRQAPGQSLEWMGDINPNNAGTSYNHKFKGRVTVTVDKSISTAYMELSRLRSDDTAVYYCVKWGDGPFAYWGQGTLVTVSS

SEQ ID NO: 57 - protein, 117 aa, synthetic construct; identical to SEQ ID NO: 56
  REGION 1..117: note = Synthetic

SEQ ID NO: 58 - protein, 117 aa, synthetic construct
  REGION 1..117: note = Synthetic
QVQLVQSGAEVKKPGASVKVSCKASGYVFTDYYMNWVRQAPGQSLEWMGDINPNNAQTQYNHKFKGRVTVTVDKSISTAYMELSRLRSDDTAVYYCVKWGDGPFAYWGQGTLVTVSS

SEQ ID NO: 59 - protein, 117 aa, synthetic construct
  REGION 1..117: note = Synthetic
QVQLVQSGAEVKKPGASVKVSCKASGYVFTDYYMNWVRQAPGQSLEWMGDINPNNAETLYNHKFKGRVTVTVDKSISTAYMELSRLRSDDTAVYYCVKWGDGPFAYWGQGTLVTVSS

SEQ ID NO: 60 - protein, 117 aa, synthetic construct
  REGION 1..117: note = Synthetic
QVQLVQSGAEVKKPGASVKVSCKASGYVFTDYYMNWVRQAPGQSLEWMGDINPNNAQTVYNHKFKGRVTVTVDKSISTAYMELSRLRSDDTAVYYCVKWGDGPFAYWGQGTLVTVSS

SEQ ID NO: 61 - protein, 106 aa, synthetic construct; identical to SEQ ID NO: 54
  REGION 1..106: note = Synthetic

SEQ ID NO: 62 - protein, 106 aa, synthetic construct
  REGION 1..106: note = Synthetic
DIQMTQSPSSLSASVGDRVTITCKASQNVKGAVAWYQQKPGKAPKLLIYSASNRYTGVPSRFSGSGSGTDFTLTISSLQPEDIATYYCQQYSNYPTFGQGTKLEIK

SEQ ID NO: 63 - protein, 106 aa, synthetic construct
  REGION 1..106: note = Synthetic
DIQMTQSPSSLSASVGDRVTITCKASQNVPAAVAWYQQKPGKAPKLLIYSASNRYTGVPSRFSGSGSGTDFTLTISSLQPEDIATYYCQQYSNYPTFGQGTKLEIK

SEQ ID NO: 64 - protein, 106 aa, synthetic construct
  REGION 1..106: note = Synthetic
DIQMTQSPSSLSASVGDRVTITCKASQNVGAAVAWYQQKPGKAPKLLIYSVSDRYTGVPSRFSGSGSGTDFTLTISSLQPEDIATYYCQQYSNYPTFGQGTKLEIK

SEQ ID NO: 65 - protein, 106 aa, synthetic construct
  REGION 1..106: note = Synthetic
DIQMTQSPSSLSASVGDRVTITCKASQNVGAAVAWYQQKPGKAPKLLIYSRSVRYTGVPSRFSGSGSGTDFTLTISSLQPEDIATYYCQQYSNYPTFGQGTKLEIK

SEQ ID NO: 66 - protein, 117 aa, synthetic construct
  REGION 1..117: note = Synthetic
GAVKFPQLCKFCDVRFSTCDNQKSCMSNCSITSICEKPQEVCVAVWRKNDENITLETVCHDPKLPYHDFILEDAASPKCIMKEKKKPGETFFMCSCSSDECNDNIIFSEEYNTSNPD

SEQ ID NO: 67 - protein, 144 aa, synthetic construct
  REGION 1..144: note = Synthetic
KMQAFRIWDVNQKTFYLRNNQLVAGYLQGPNVNLEEKIDVVPIEPHALFLGIHGGKMCLSCVKSGDETRLQLEAVNITDLSENRKQDKRFAFIRSDSGPTTSFESAACPGWFLCTAMEADQPVSLTNMPDEGVMVTKFYFQEDE

SEQ ID NO: 68 - protein, 21 aa, synthetic construct
  REGION 1..21: note = Synthetic
GGGGSGGGGSGGGGSGGGGSG

SEQ ID NO: 69 - protein, 470 aa, Homo sapiens
LQCFCHLCTKDNFTCVTDGLCFVSVTETTDKVIHNSMCIAEIDLIPRDRPFVCAPSSKTGSVTTTYCCNQDHCNKIELPTTVKSSPGLGPVELAAVIAGPVCFVCISLMLMVYICHNRTVIHHRVPNEEDPSLDRPFISEGTTLKDLIYDMTTSGSGSGLPLLVQRTIARTIVLQESIGKGRFGEVWRGKWRGEEVAVKIFSSREERSWFREAEIYQTVMLRHENILGFIAADNKDNGTWTQLWLVSDYHEHGSLFDYLNRYTVTVEGMIKLALSTASGLAHLHMEIVGTQGKPAIAHRDLKSKNILVKKNGTCCIADLGLAVRHDSATDTIDIAPNHRVGTKRYMAPEVLDDSINMKHFESFKRADIYAMGLVFWEIARRCSIGGIHEDYQLPYYDLVPSDPSVEEMRKVVCEQKLRPNIPNRWQSCEALRVMAKIMRECWYANGAARLTALRIKKTLSQLSQQEGIKM

SEQ ID NO: 70 - protein, 545 aa, Homo sapiens
TIPPHVQKSVNNDMIVTDNNGAVKFPQLCKFCDVRFSTCDNQKSCMSNCSITSICEKPQEVCVAVWRKNDENITLETVCHDPKLPYHDFILEDAASPKCIMKEKKKPGETFFMCSCSSDECNDNIIFSEEYNTSNPDLLLVIFQVTGISLLPPLGVAISVIIIFYCYRVNRQQKLSSTWETGKTRKLMEFSEHCAIILEDDRSDISSTCANNINHNTELLPIELDTLVGKGRFAEVYKAKLKQNTSEQFETVAVKIFPYEEYASWKTEKDIFSDINLKHENILQFLTAEERKTELGKQYWLITAFHAKGNLQEYLTRHVISWEDLRKLGSSLARGIAHLHSDHTPCGRPKMPIVHRDLKSSNILVKNDLTCCLCDFGLSLRLDPTLSVDDLANSGQVGTARYMAPEVLESRMNLENVESFKQTDVYSMALVLWEMTSRCNAVGEVKDYEPPFGSKVREHPCVESMKDNVLRDRGRPEIPSFWLNHQGIQMVCETLTECWDHDPEARLTAQCVAERFSELEHLDRLSGRSCSEEKIPEDGSLNTTK

SEQ ID NO: 71 - protein, 570 aa, Homo sapiens
TIPPHVQKSDVEMEAQKDEIICPSCNRTAHPLRHINNDMIVTDNNGAVKFPQLCKFCDVRFSTCDNQKSCMSNCSITSICEKPQEVCVAVWRKNDENITLETVCHDPKLPYHDFILEDAASPKCIMKEKKKPGETFFMCSCSSDECNDNIIFSEEYNTSNPDLLLVIFQVTGISLLPPLGVAISVIIIFYCYRVNRQQKLSSTWETGKTRKLMEFSEHCAIILEDDRSDISSTCANNINHNTELLPIELDTLVGKGRFAEVYKAKLKQNTSEQFETVAVKIFPYEEYASWKTEKDIFSDINLKHENILQFLTAEERKTELGKQYWLITAFHAKGNLQEYLTRHVISWEDLRKLGSSLARGIAHLHSDHTPCGRPKMPIVHRDLKSSNILVKNDLTCCLCDFGLSLRLDPTLSVDDLANSGQVGTARYMAPEVLESRMNLENVESFKQTDVYSMALVLWEMTSRCNAVGEVKDYEPPFGSKVREHPCVESMKDNVLRDRGRPEIPSFWLNHQGIQMVCETLTECWDHDPEARLTAQCVAERFSELEHLDRLSGRSCSEEKIPEDGSLNTTK

SEQ ID NO: 72 - protein, 831 aa, Homo sapiens
GPEPGALCELSPVSASHPVQALMESFTVLSGCASRGTTGLPQEVHVLNLRTAGQGPGQLQREVTLHLNPISSVHIHHKSVVFLLNSPHPLVWHLKTERLATGVSRLFLVSEGSVVQFSSANFSLTAETEERNFPHGNEHLLNWARKEYGAVTSFTELKIARNIYIKVGEDQVFPPKCNIGKNFLSLNYLAEYLQPKAAEGCVMSSQPQNEEVHIIELITPNSNPYSAFQVDITIDIRPSQEDLEVVKNLILILKCKKSVNWVIKSFDVKGSLKIIAPNSIGFGKESERSMTMTKSIRDDIPSTQGNLVKWALDNGYSPITSYTMAPVANRFHLRLENNAEEMGDEEVHTIPPELRILLDPGALPALQNPPIRGGEGQNGGLPFPFPDISRRVWNEEGEDGLPRPKDPVIPSIQLFPGLREPEEVQGSVDIALSVKCDNEKMIVAVEKDSFQASGYSGMDVTLLDPTCKAKMNGTHFVLESPLNGCGTRPRWSALDGVVYYNSIVIQVPALGDSSGWPDGYEDLESGDNGFPGDMDEGDASLFTRPEIVVFNCSLQQVRNPSSFQEQPHGNITFNMELYNTDLFLVPSQGVFSVPENGHVYVEVSVTKAEQELGFAIQTCFISPYSNPDRMSHYTIIENICPKDESVKFYSPKRVHFPIPQADMDKKRFSFVFKPVFNTSLLFLQCELTLCTKMEKHPQKLPKCVPPDEACTSLDASIIWAMMQNKKTFTKPLAVIHHEAESKEKGPSMKEPNPISPPIFHGLDTLTVMGIAFAAFVIGALLTGALWYIYSHTGETAGRQQVPTSPPASENSSAAHSIGSTQSTPCSSSSTA

SEQ ID NO: 73 - protein, 552 aa, Homo sapiens
LEADKCKEREEKIILVSSANEIDVRPCPLNPNEHKGTITWYKDDSKTPVSTEQASRIHQHKEKLWFVPAKVEDSGHYYCVVRNSSYCLRIKISAKFVENEPNLCYNAQAIFKQKLPVAGDGGLVCPYMEFFKNENNELPKLQWYKDCKPLLLDNIHFSGVKDRLIVMNVAEKHRGNYTCHASYTYLGKQYPITRVIEFITLEENKPTRPVIVSPANETMEVDLGSQIQLICNVTGQLSDIAYWKWNGSVIDEDDPVLGEDYYSVENPANKRRSTLITVLNISEIESRFYKHPFTCFAKNTHGIDAAYIQLIYPVTNFQKHMIGICVTLTVIIVCSVFIYKIFKIDIVLWYRDSCYDFLPIKASDGKTYDAYILYPKTVGEGSTSDCDIFVFKVLPEVLEKQCGYKLFIYGRDDYVGEDIVEVINENVKKSRRLIIILVRETSGFSWLGGSSEEQIAMYNALVQDGIKVVLLELEKIQDYEKMPESIKFIKQKHGAIRWSGDFTQGPQSAKTRFWKNVRYHMPVQRRSPSSKHQLLSPATKEKLQREAHVPLG

SEQ ID NO: 74 - protein, 550 aa, Homo sapiens
SERCDDWGLDTMRQIQVFEDEPARIKCPLFEHFLKFNYSTAHSAGLTLIWYWTRQDRDLEEPINFRLPENRISKEKDVLWFRPTLLNDTGNYTCMLRNTTYCSKVAFPLEVVQKDSCFNSPMKLPVHKLYIEYGIQRITCPNVDGYFPSSVKPTITWYMGCYKIQNFNNVIPEGMNLSFLIALISNNGNYTCVVTYPENGRTFHLTRTLTVKVVGSPKNAVPPVIHSPNDHVVYEKEPGEELLIPCTVYFSFLMDSRNEVWWTIDGKKPDDITIDVTINESISHSRTEDETRTQILSIKKVTSEDLKRSYVCHARSAKGEVAKAAKVKQKVPAPRYTVELACGFGATVLLVVILIVVYHVYWLEMVLFYRAHFGTDETILDGKEYDIYVSYARNAEEEEFVLLTLRGVLENEFGYKLCIFDRDSLPGGIVTDETLSFIQKSRRLLVVLSPNYVLQGTQALLELKAGLENMASRGNINVILVQYKAVKETKVKELKRAKTVLTVIKWKGEKSKYPQGRFWKQLQVAMPVKKSPRRSSSDEQGLSYSSLKNV

SEQ ID NO: 75 - protein, 385 aa, Homo sapiens
FTLQPAAHTGAARSCRFRGRHYKREFRLEGEPVALRCPQVPYWLWASVSPRINLTWHKNDSARTVPGEEETRMWAQDGALWLLPALQEDSGTYVCTTRNASYCDKMSIELRVFENTDAFLPFISYPQILTLSTSGVLVCPDLSEFTRDKTDVKIQWYKDSLLLDKDNEKFLSVRGTTHLLVHDVALEDAGYYRCVLTFAHEGQQYNITRSIELRIKKKKEETIPVIISPLKTISASLGSRLTIPCKVFLGTGTPLTTMLWWTANDTHIESAYPGGRVTEGPRQEYSENNENYIEVPLIFDPVTREDLHMDFKCVVHNTLSFQTLRTTVKEASSTFSWGIVLAPLSLAFLVLGGIWMHRRCKHRTGKADGLTVLWPHHQDFQSYPK

SEQ ID NO: 76 - protein, 152 aa, Homo sapiens
RPSGRKSSKMQAFRIWDVNQKTFYLRNNQLVAGYLQGPNVNLEEKIDVVPIEPHALFLGIHGGKMCLSCVKSGDETRLQLEAVNITDLSENRKQDKRFAFIRSDSGPTTSFESAACPGWFLCTAMEADQPVSLTNMPDEGVMVTKFYFQEDE

SEQ ID NO: 77 - protein, 93 aa, synthetic construct
  REGION 1..93: note = Synthetic
LQCFCHLCTKDNFTCVTDGLCFVSVTETTDKVIHNSMCIAEIDLIPRDRPFVCAPSSKTGSVTTTYCCNQDHCNKIELPTTVKSSPGLGPVEL

SEQ ID NO: 78 - protein, 136 aa, synthetic construct
  REGION 1..136: note = Synthetic
IPPHVQKSVNNDMIVTDNNGAVKFPQLCKFCDVRFSTCDNQKSCMSNCSITSICEKPQEVCVAVWRKNDENITLETVCHDPKLPYHDFILEDAASPKCIMKEKKKPGETFFMCSCSSDECNDNIIFSEEYNTSNPD

SEQ ID NO: 79 - protein, 767 aa, synthetic construct
  REGION 1..767: note = Synthetic
GPEPGALCELSPVSASHPVQALMESFTVLSGCASRGTTGLPQEVHVLNLRTAGQGPGQLQREVTLHLNPISSVHIHHKSVVFLLNSPHPLVWHLKTERLATGVSRLFLVSEGSVVQFSSANFSLTAETEERNFPHGNEHLLNWARKEYGAVTSFTELKIARNIYIKVGEDQVFPPKCNIGKNFLSLNYLAEYLQPKAAEGCVMSSQPQNEEVHIIELITPNSNPYSAFQVDITIDIRPSQEDLEVVKNLILILKCKKSVNWVIKSFDVKGSLKIIAPNSIGFGKESERSMTMTKSIRDDIPSTQGNLVKWALDNGYSPITSYTMAPVANRFHLRLENNAEEMGDEEVHTIPPELRILLDPGALPALQNPPIRGGEGQNGGLPFPFPDISRRVWNEEGEDGLPRPKDPVIPSIQLFPGLREPEEVQGSVDIALSVKCDNEKMIVAVEKDSFQASGYSGMDVTLLDPTCKAKMNGTHFVLESPLNGCGTRPRWSALDGVVYYNSIVIQVPALGDSSGWPDGYEDLESGDNGFPGDMDEGDASLFTRPEIVVFNCSLQQVRNPSSFQEQPHGNITFNMELYNTDLFLVPSQGVFSVPENGHVYVEVSVTKAEQELGFAIQTCFISPYSNPDRMSHYTIIENICPKDESVKFYSPKRVHFPIPQADMDKKRFSFVFKPVFNTSLLFLQCELTLCTKMEKHPQKLPKCVPPDEACTSLDASIIWAMMQNKKTFTKPLAVIHHEAESKEKGPSMKEPNPISPPIFHGLDTLTV

SEQ ID NO: 80 - protein, 330 aa, synthetic construct [sequence omitted]

SEQ ID NO: 81 - protein, 330 aa, synthetic construct
  REGION 1..330: note = Synthetic
ASTKGPSVFPLAPSSKSTSGGTAALGCLVKDYFPEPVTVSWNSGALTSGVHTFPAVLQSSGLYSLSSVVTVPSSSLGTQTYICNVNHKPSNTKVDKKVEPKSCDKTHTCPPCPAPEFEGGPSVFLFPPKPKDTLMISRTPEVTCVVVDVSHEDPEVKFNWYVDGVEVHNAKTKPREEQYNSTYRVVSVLTVLHQDWLNGKEYKCKVSNKALPASIEKTISKAKGQPREPQVYTLPPSRDELTKNQVSLTCLVKGFYPSDIAVEWESNGQPENNYKTTPPVLDSDGSFFLYSKLTVDKSRWQQGNVFSCSVMHEALHNHYTQKSLSLSPGA

SEQ ID NO: 82 - protein, 107 aa, synthetic construct [sequence omitted]

SEQ ID NO: 83 - protein, 330 aa, synthetic construct; identical to SEQ ID NO: 81
  REGION 1..330: note = Synthetic

SEQ ID NO: 84 - protein, 119 aa, synthetic construct
  REGION 1..119: note = Synthetic
EEELQIIQPDKSVLVAAGETATLRCTITSLFPVGPIQWFRGAGPGRVLIYNQRQGPFPRVTTVSDTTKRNNMDFSIRIGNITPADAGTYYCIKFRKGSPDDVEFKSGAGTELSVRAKPS

SEQ ID NO: 85 - protein, 107 aa, synthetic construct [sequence omitted]

SEQ ID NO: 86 - protein, 118 aa, synthetic construct [sequence omitted]

SEQ ID NO: 87 - protein, 330 aa, synthetic construct
  REGION 1..330: note = Synthetic
ASTKGPSVFPLAPSSKSTSGGTAALGCLVKDYFPEPVTVSWNSGALTSGVHTFPAVLQSSGLYSLSSVVTVPSSSLGTQTYICNVNHKPSNTKVDKKVEPKSCDKTHTCPPCPAPELLGGPSVFLFPPKPKDTLMISRTPEVTCVVVDVSHEDPEVKFNWYVDGVEVHNAKTKPREEQYASTYRVVSVLTVLHQDWLNGKEYKCKVSNKALPAPIEKTISKAKGQPREPQVYTLPPSREEMTKNQVSLTCLVKGFYPSDIAVEWESNGQPENNYKTTPPVLDSDGSFFLYSKLTVDKSRWQQGNVFSCSVMHEALHNHYTQKSLSLSPGA

SEQ ID NO: 88 - protein, 330 aa, synthetic construct
  REGION 1..330: note = Synthetic
ASTKGPSVFPLAPSSKSTSGGTAALGCLVKDYFPEPVTVSWNSGALTSGVHTFPAVLQSSGLYSLSSVVTVPSSSLGTQTYICNVNHKPSNTKVDKKVEPKSCDKTHTCPPCPAPEFEGGPSVFLFPPKPKDTLMISRTPEVTCVVVDVSHEDPEVKFNWYVDGVEVHNAKTKPREEQYNSTYRVVSVLTVLHQDWLNGKEYKCKVSNKALPASIEKTISKAKGQPREPQVYTLPPCRDELTKNQVSLWCLVKGFYPSDIAVEWESNGQPENNYKTTPPVLDSDGSFFLYSKLTVDKSRWQQGNVFSCSVMHEALHNHYTQKSLSLSPGA

SEQ ID NO: 89 - protein, 330 aa, synthetic construct
  REGION 1..330: note = Synthetic
ASTKGPSVFPLAPSSKSTSGGTAALGCLVKDYFPEPVTVSWNSGALTSGVHTFPAVLQSSGLYSLSSVVTVPSSSLGTQTYICNVNHKPSNTKVDKKVEPKSCDKTHTCPPCPAPEFEGGPSVFLFPPKPKDTLMISRTPEVTCVVVDVSHEDPEVKFNWYVDGVEVHNAKTKPREEQYNSTYRVVSVLTVLHQDWLNGKEYKCKVSNKALPASIEKTISKAKGQPREPQVCTLPPSRDELTKNQVSLSCAVKGFYPSDIAVEWESNGQPENNYKTTPPVLDSDGSFFLVSKLTVDKSRWQQGNVFSCSVMHEALHNHYTQKSLSLSPGK

SEQ ID NO: 90 - protein, 213 aa, synthetic construct
  REGION 1..213: note = Synthetic
DIQMTQSPSSLSASVGDRVTITCKASQNVGAAVAWYQQKPGKAPKLLIYSVSDRYTGVPSRFSGSGSGTDFTLTISSLQPEDIATYYCQQYSNYPTFGQGTKLEIKRTVAAPSVFIFPPSDEQLKSGTASVVCLLNNFYPREAKVQWKVDNALQSGNSQESVTEQDSKDSTYSLSSTLTLSKADYEKHKVYACEVTHQGLSSPVTKSFNRGEC

SEQ ID NO: 91 - protein, 587 aa, synthetic construct
  REGION 1..587: note = Synthetic
QVQLVQSGAEVKKPGASVKVSCKASGYVFTDYYMNWVRQAPGQSLEWMGDINPNNAETLYNHKFKGRVTVTVDKSISTAYMELSRLRSDDTAVYYCVKWGDGPFAYWGQGTLVTVSSASTKGPSVFPLAPSSKSTSGGTAALGCLVKDYFPEPVTVSWNSGALTSGVHTFPAVLQSSGLYSLSSVVTVPSSSLGTQTYICNVNHKPSNTKVDKKVEPKSCDKTHTCPPCPAPEFEGGPSVFLFPPKPKDTLMISRTPEVTCVVVDVSHEDPEVKFNWYVDGVEVHNAKTKPREEQYNSTYRVVSVLTVLHQDWLNGKEYKCKVSNKALPASIEKTISKAKGQPREPQVYTLPPSRDELTKNQVSLTCLVKGFYPSDIAVEWESNGQPENNYKTTPPVLDSDGSFFLYSKLTVDKSRWQQGNVFSCSVMHEALHNHYTQKSLSLSPGAGGGGSGGGGSGGGGSGGGGSGEEELQIIQPDKSVLVAAGETATLRCTITSLFPVGPIQWFRGAGPGRVLIYNQRQGPFPRVTTVSDTTKRNNMDFSIRIGNITPADAGTYYCIKFRKGSPDDVEFKSGAGTELSVRAKPS

SEQ ID NO: 92 - protein, 214 aa, synthetic construct
  REGION 1..214: note = Synthetic
DIQMTQSPSSLSASVGDRVTITCRASQDVSTAVAWYQQKPGKAPKLLIYSASFLYSGVPSRFSGSGSGTDFTLTISSLQPEDFATYYCQQYLYHPATFGQGTKVEIKRTVAAPSVFIFPPSDEQLKSGTASVVCLLNNFYPREAKVQWKVDNALQSGNSQESVTEQDSKDSTYSLSSTLTLSKADYEKHKVYACEVTHQGLSSPVTKSFNRGEC

SEQ ID NO: 93 - protein, 588 aa, synthetic construct
  REGION 1..588: note = Synthetic
EVQLVESGGGLVQPGGSLRLSCAASGFTFSDSWIHWVRQAPGKGLEWVAWISPYGGSTYYADSVKGRFTISADTSKNTAYLQMNSLRAEDTAVYYCARRHWPGGFDYWGQGTLVTVSSASTKGPSVFPLAPSSKSTSGGTAALGCLVKDYFPEPVTVSWNSGALTSGVHTFPAVLQSSGLYSLSSVVTVPSSSLGTQTYICNVNHKPSNTKVDKKVEPKSCDKTHTCPPCPAPELLGGPSVFLFPPKPKDTLMISRTPEVTCVVVDVSHEDPEVKFNWYVDGVEVHNAKTKPREEQYNSTYRVVSVLTVLHQDWLNGKEYKCKVSNKALPAPIEKTISKAKGQPREPQVYTLPPSREEMTKNQVSLTCLVKGFYPSDIAVEWESNGQPENNYKTTPPVLDSDGSFFLYSKLTVDKSRWQQGNVFSCSVMHEALHNHYTQKSLSLSPGAGGGGSGGGGSGGGGSGGGGSGEEELQIIQPDKSVLVAAGETATLRCTITSLFPVGPIQWFRGAGPGRVLIYNQRQGPFPRVTTVSDTTKRNNMDFSIRIGNITPADAGTYYCIKFRKGSPDDVEFKSGAGTELSVRAKPS

SEQ ID NO: 94 - protein, 587 aa, synthetic construct
  REGION 1..587: note = Synthetic
QVQLVQSGAEVKKPGASVKVSCKASGYVFTDYYMNWVRQAPGQSLEWMGDINPNNAETLYNHKFKGRVTVTVDKSISTAYMELSRLRSDDTAVYYCVKWGDGPFAYWGQGTLVTVSSASTKGPSVFPLAPSSKSTSGGTAALGCLVKDYFPEPVTVSWNSGALTSGVHTFPAVLQSSGLYSLSSVVTVPSSSLGTQTYICNVNHKPSNTKVDKKVEPKSCDKTHTCPPCPAPEFEGGPSVFLFPPKPKDTLMISRTPEVTCVVVDVSHEDPEVKFNWYVDGVEVHNAKTKPREEQYNSTYRVVSVLTVLHQDWLNGKEYKCKVSNKALPASIEKTISKAKGQPREPQVYTLPPCRDELTKNQVSLWCLVKGFYPSDIAVEWESNGQPENNYKTTPPVLDSDGSFFLYSKLTVDKSRWQQGNVFSCSVMHEALHNHYTQKSLSLSPGAGGGGSGGGGSGGGGSGGGGSGEEELQIIQPDKSVLVAAGETATLRCTITSLFPVGPIQWFRGAGPGRVLIYNQRQGPFPRVTTVSDTTKRNNMDFSIRIGNITPADAGTYYCIKFRKGSPDDVEFKSGAGTELSVRAKPS

SEQ ID NO: 95 - protein, 447 aa, synthetic construct
  REGION 1..447: note = Synthetic
QVQLVQSGAEVKKPGASVKVSCKASGYVFTDYYMNWVRQAPGQSLEWMGDINPNNAETLYNHKFKGRVTVTVDKSISTAYMELSRLRSDDTAVYYCVKWGDGPFAYWGQGTLVTVSSASTKGPSVFPLAPSSKSTSGGTAALGCLVKDYFPEPVTVSWNSGALTSGVHTFPAVLQSSGLYSLSSVVTVPSSSLGTQTYICNVNHKPSNTKVDKKVEPKSCDKTHTCPPCPAPEFEGGPSVFLFPPKPKDTLMISRTPEVTCVVVDVSHEDPEVKFNWYVDGVEVHNAKTKPREEQYNSTYRVVSVLTVLHQDWLNGKEYKCKVSNKALPASIEKTISKAKGQPREPQVCTLPPSRDELTKNQVSLSCAVKGFYPSDIAVEWESNGQPENNYKTTPPVLDSDGSFFLVSKLTVDKSRWQQGNVFSCSVMHEALHNHYTQKSLSLSPGK

SEQ ID NO: 96 - protein, 588 aa, synthetic construct
  REGION 1..588: note = Synthetic
EVQLVESGGGLVQPGGSLRLSCAASGFTFSDSWIHWVRQAPGKGLEWVAWISPYGGSTYYADSVKGRFTISADTSKNTAYLQMNSLRAEDTAVYYCARRHWPGGFDYWGQGTLVTVSSASTKGPSVFPLAPSSKSTSGGTAALGCLVKDYFPEPVTVSWNSGALTSGVHTFPAVLQSSGLYSLSSVVTVPSSSLGTQTYICNVNHKPSNTKVDKKVEPKSCDKTHTCPPCPAPEFEGGPSVFLFPPKPKDTLMISRTPEVTCVVVDVSHEDPEVKFNWYVDGVEVHNAKTKPREEQYNSTYRVVSVLTVLHQDWLNGKEYKCKVSNKALPASIEKTISKAKGQPREPQVYTLPPCRDELTKNQVSLWCLVKGFYPSDIAVEWESNGQPENNYKTTPPVLDSDGSFFLYSKLTVDKSRWQQGNVFSCSVMHEALHNHYTQKSLSLSPGAGGGGSGGGGSGGGGSGGGGSGEEELQIIQPDKSVLVAAGETATLRCTITSLFPVGPIQWFRGAGPGRVLIYNQRQGPFPRVTTVSDTTKRNNMDFSIRIGNITPADAGTYYCIKFRKGSPDDVEFKSGAGTELSVRAKPS

SEQ ID NO: 97 - protein, 448 aa, synthetic construct
  REGION 1..448: note = Synthetic
EVQLVESGGGLVQPGGSLRLSCAASGFTFSDSWIHWVRQAPGKGLEWVAWISPYGGSTYYADSVKGRFTISADTSKNTAYLQMNSLRAEDTAVYYCARRHWPGGFDYWGQGTLVTVSSASTKGPSVFPLAPSSKSTSGGTAALGCLVKDYFPEPVTVSWNSGALTSGVHTFPAVLQSSGLYSLSSVVTVPSSSLGTQTYICNVNHKPSNTKVDKKVEPKSCDKTHTCPPCPAPEFEGGPSVFLFPPKPKDTLMISRTPEVTCVVVDVSHEDPEVKFNWYVDGVEVHNAKTKPREEQYNSTYRVVSVLTVLHQDWLNGKEYKCKVSNKALPASIEKTISKAKGQPREPQVCTLPPSRDELTKNQVSLSCAVKGFYPSDIAVEWESNGQPENNYKTTPPVLDSDGSFFLVSKLTVDKSRWQQGNVFSCSVMHEALHNHYTQKSLSLSPGK

SEQ ID NO: 98 - protein, 119 aa, synthetic construct
  REGION 1..119: note = Synthetic
EEELQVIQPDKSVLVAAGETATLRCTVTSLIPVGPIQWFRGAGPGRELIYNQKEGHFPRVTTVSDSTKRNNMDFSIRIGNITPADAGTYYCVKFRKGSPDDVEFKSGAGTELSVRAKPS

SEQ ID NO: 99 - protein, 150 aa, synthetic construct
  REGION 1..150: note = Synthetic
LQPGAEVPVVWAQEGAPAQLPCSPTIPLQDLSLLRRAGVTWQHQPDSGPPAAAPGHPLAPGPHPAAPSSWGPRPRRYTVLSVGPGGLRSGRLPLQPRVQLDERGRQRGDFSLWLRPARRADAGEYRAAVHLRDRALSCRLRLRLGQASMT

SEQ ID NO: 100 - protein, 260 aa, synthetic construct
  REGION 1..260: note = Synthetic
LQPGAEVPVVWAQEGAPAQLPCSPTIPLQDLSLLRRAGVTWQHQPDSGPPAAAPGHPLAPGPHPAAPSSWGPRPRRYTVLSVGPGGLRSGRLPLQPRVQLDERGRQRGDFSLWLRPARRADAGEYRAAVHLRDRALSCRLRLRLGQASMTASPPGSLRASDWVILNCSFSRPDRPASVHWFRNRGQGRVPVRESPHHHLAESFLFLPQVSPMDSGPWGCILTYRDGFNVSIMYNLTVLGLEPPTPLTVYAGAGSRVGLPC

SEQ ID NO: 101 - protein, 29 aa, synthetic construct
  REGION 1..29: note = Synthetic
GPPAAAPGHPLAPGPHPAAPSSWGPRPRR

SEQ ID NO: 102 - protein, 120 aa, synthetic construct [sequence omitted]

SEQ ID NO: 103 - protein, 107 aa, synthetic construct [sequence omitted]

SEQ ID NO: 104 - protein, 7 aa, synthetic construct
  REGION 1..7: note = Synthetic
TSGMGVG

SEQ ID NO: 105 - protein, 16 aa, synthetic construct
  REGION 1..16: note = Synthetic
HIWWDGDESYNPSLKS

SEQ ID NO: 106 - protein, 10 aa, synthetic construct
  REGION 1..10: note = Synthetic
NRYDPPWFVD

SEQ ID NO: 107 - protein, 11 aa, synthetic construct
  REGION 1..11: note = Synthetic
RASQDISNYLS

SEQ ID NO: 108 - protein, 7 aa, synthetic construct
  REGION 1..7: note = Synthetic
YTSKLHS

SEQ ID NO: 109 - protein, 9 aa, synthetic construct
  REGION 1..9: note = Synthetic
LQGKMLPWT

SEQ ID NO: 110 - protein, 118 aa, synthetic construct [sequence omitted]

SEQ ID NO: 111 - protein, 107 aa, synthetic construct [sequence omitted]

SEQ ID NO: 112 - protein, 5 aa, synthetic construct
  REGION 1..5: note = Synthetic
VYGMN

SEQ ID NO: 113 - protein, 17 aa, synthetic construct
  REGION 1..17: note = Synthetic
IIWYDGDNQYYADSVKG

SEQ ID NO: 114 - protein, 9 aa, synthetic construct
  REGION 1..9: note = Synthetic
DLRTGPFDY

SEQ ID NO: 115 - protein, 11 aa, synthetic construct
  REGION 1..11: note = Synthetic
RASQSIGSSLH

SEQ ID NO: 116 - protein, 7 aa, synthetic construct
  REGION 1..7: note = Synthetic
YASQSFS

SEQ ID NO: 117 - protein, 9 aa, synthetic construct
  REGION 1..9: note = Synthetic
HQSSSLPFT

SEQ ID NO: 118 - protein, 713 aa, synthetic construct
  REGION 1..713: note = Synthetic
QVQLQESGPGLVKPSQTLSLTCSFSGFSLSTSGMGVGWIRQPSGKGLEWLAHIWWDGDESYNPSLKSRLTISKDTSKNQVSLKITSVTAADTAVYFCARNRYDPPWFVDWGQGTLVTVSSASTKGPSVFPLAPSSKSTSGGTAALGCLVKDYFPEPVTVSWNSGALTSGVHTFPAVLQSSGLYSLSSVVTVPSSSLGTQTYICNVNHKPSNTKVDKKVEPKSCDKTHTCPPCPAPEFEGGPSVFLFPPKPKDTLMISRTPEVTCVVVDVSHEDPEVKFNWYVDGVEVHNAKTKPREEQYNSTYRVVSVLTVLHQDWLNGKEYKCKVSNKALPASIEKTISKAKGQPREPQVYTLPPSRDELTKNQVSLTCLVKGFYPSDIAVEWESNGQPENNYKTTPPVLDSDGSFFLYSKLTVDKSRWQQGNVFSCSVMHEALHNHYTQKSLSLSPGAGGGGSGGGGSGGGGSGGGGSQVQLVQSGAEVKKPGASVKVSCKASGYVFTDYYMNWVRQAPGQSLEWMGDINPNNAETLYNHKFKGRVTVTVDKSISTAYMELSRLRSDDTAVYYCVKWGDGPFAYWGQGTLVTVSSGGGGSGGGGSGGGGSGGGGSDIQMTQSPSSLSASVGDRVTITCKASQNVGAAVAWYQQKPGKAPKLLIYSVSDRYTGVPSRFSGSGSGTDFTLTISSLQPEDIATYYCQQYSNYPTFGQGTKLTVL

SEQ ID NO: 119 - protein, 214 aa, synthetic construct
  REGION 1..214: note = Synthetic
DIQMTQSTSSLSASVGDRVTITCRASQDISNYLSWYQQKPGKAVKLLIYYTSKLHSGVPSRFSGSGSGTDYTLTISSLQQEDFATYFCLQGKMLPWTFGQGTKLEIKRTVAAPSVFIFPPSDEQLKSGTASVVCLLNNFYPREAKVQWKVDNALQSGNSQESVTEQDSKDSTYSLSSTLTLSKADYEKHKVYACEVTHQGLSSPVTKSFNRGEC

SEQ ID NO: 120 - protein, 711 aa, synthetic construct
  REGION 1..711: note = Synthetic
QVQLVESGGGVVQPGRSLRLSCAASGFTFSVYGMNWVRQAPGKGLEWVAIIWYDGDNQYYADSVKGRFTISRDNSKNTLYLQMNGLRAEDTAVYYCARDLRTGPFDYWGQGTLVTVSSASTKGPSVFPLAPSSKSTSGGTAALGCLVKDYFPEPVTVSWNSGALTSGVHTFPAVLQSSGLYSLSSVVTVPSSSLGTQTYICNVNHKPSNTKVDKKVEPKSCDKTHTCPPCPAPEFEGGPSVFLFPPKPKDTLMISRTPEVTCVVVDVSHEDPEVKFNWYVDGVEVHNAKTKPREEQYNSTYRVVSVLTVLHQDWLNGKEYKCKVSNKALPASIEKTISKAKGQPREPQVYTLPPSRDELTKNQVSLTCLVKGFYPSDIAVEWESNGQPENNYKTTPPVLDSDGSFFLYSKLTVDKSRWQQGNVFSCSVMHEALHNHYTQKSLSLSPGAGGGGSGGGGSGGGGSGGGGSQVQLVQSGAEVKKPGASVKVSCKASGYVFTDYYMNWVRQAPGQCLEWMGDINPNNAETLYNHKFKGRVTVTVDKSISTAYMELSRLRSDDTAVYYCVKWGDGPFAYWGQGTLVTVSSGGGGSGGGGSGGGGSGGGGSDIQMTQSPSSLSASVGDRVTITCKASQNVGAAVAWYQQKPGKAPKLLIYSVSDRYTGVPSRFSGSGSGTDFTLTISSLQPEDIATYYCQQYSNYPTFGCGTKLTVL

SEQ ID NO: 121 - protein, 214 aa, synthetic construct
  REGION 1..214: note = Synthetic
EIVLTQSPDFQSVTPKEKVTITCRASQSIGSSLHWYQQKPDQSPKLLIKYASQSFSGVPSRFSGSGSGTDFTLTINSLEAEDAAAYYCHQSSSLPFTFGPGTKVDIKRTVAAPSVFIFPPSDEQLKSGTASVVCLLNNFYPREAKVQWKVDNALQSGNSQESVTEQDSKDSTYSLSSTLTLSKADYEKHKVYACEVTHQGLSSPVTKSFNRGEC

SEQ ID NO: 122 - protein, 20 aa, synthetic construct
  REGION 1..20: note = synthetic
GGGGSGGGGSGGGGSGGGGS